European Patent Specification EP 3 269 813 B1, published May 24, 2023. Title: A method for isolating nucleic acid from FFPE tissue. Applicant: THE ASAN FOUNDATION University of Ulsan Foundation For Industry Cooperation. The sequence listing filed with the application follows.

SEQUENCE LISTING (120 sequences)

SEQ ID NO: 1 - DNA, 30 bp, Artificial Sequence
  rs248205-2nd
acgttggatgggctcatgggaagaatcatc

SEQ ID NO: 2 - DNA, 29 bp, Artificial Sequence
  rs248205-1st
acgttggatggggcaacataccactattg

SEQ ID NO: 3 - DNA, 30 bp, Artificial Sequence
  rs2051068-2nd
acgttggatgaccctggaaaccatttcaga

SEQ ID NO: 4 - DNA, 29 bp, Artificial Sequence
  rs2051068-1st
acgttggatgctgaaggtaaagattcaag

SEQ ID NO: 5 - DNA, 30 bp, Artificial Sequence
  rs1950501-2nd
acgttggatgaatgactcaccactgaccac

SEQ ID NO: 6 - DNA, 30 bp, Artificial Sequence
  rs1950501-1st
acgttggatgtgttgtctgggaactcaggg

SEQ ID NO: 7 - DNA, 30 bp, Artificial Sequence
  rs1952966-2nd
acgttggatgggctctggttacaacagctt

SEQ ID NO: 8 - DNA, 30 bp, Artificial Sequence
  rs1952966-1st
acgttggatgagaagtttgcttggctgaag

SEQ ID NO: 9 - DNA, 30 bp, Artificial Sequence
  AMG_mid100-2nd
acgttggatgggcttgaggccaaccatcag

SEQ ID NO: 10 - DNA, 30 bp, Artificial Sequence
  AMG_mid100-1st
acgttggatgcctcatcctgggcaccctgg

SEQ ID NO: 11 - DNA, 30 bp, Artificial Sequence
  rs1385306-2nd
acgttggatggtctgtcagctgttctgatg

SEQ ID NO: 12 - DNA, 30 bp, Artificial Sequence; identical to SEQ ID NO: 9
  rs1385306-1st

SEQ ID NO: 13 - DNA, 30 bp, Artificial Sequence
  rs1365740-2nd
acgttggatggtacttacctcctgaggtag

SEQ ID NO: 14 - DNA, 30 bp, Artificial Sequence
  rs1365740-1st
acgttggatgacttcctatgttgccagcac

SEQ ID NO: 15 - DNA, 30 bp, Artificial Sequence
  rs2016207-2nd
acgttggatgctgatgcaaaaatctatggc

SEQ ID NO: 16 - DNA, 30 bp, Artificial Sequence
  rs2016207-1st
acgttggatggctctagtagattgctagcc

SEQ ID NO: 17 - DNA, 30 bp, Artificial Sequence
  rs1571256-2nd
acgttggatgataccgcagaagtttggcac

SEQ ID NO: 18 - DNA, 30 bp, Artificial Sequence
  rs1571256-1st
acgttggatggcattctaaacatgcctctc

SEQ ID NO: 19 - DNA, 30 bp, Artificial Sequence
  rs1350836-2nd
acgttggatgatttcagactgttgtgctgg

SEQ ID NO: 20 - DNA, 30 bp, Artificial Sequence
  rs1350836-1st
acgttggatgcctgtggccttttcatggag

SEQ ID NO: 21 - DNA, 30 bp, Artificial Sequence
  rs120434-2nd
acgttggatgatgccttgttccatgtgctg

SEQ ID NO: 22 - DNA, 30 bp, Artificial Sequence
  rs120434-1st
acgttggatgacacaagtggaagcttgcag

SEQ ID NO: 23 - DNA, 30 bp, Artificial Sequence
  rs2347790-2nd
acgttggatgatgctccacccacacagttc

SEQ ID NO: 24 - DNA, 30 bp, Artificial Sequence
  rs2347790-1st
acgttggatgacctatgcaacagctggaag

SEQ ID NO: 25 - DNA, 31 bp, Artificial Sequence
  rs298898-2nd
acgttggatgccatatatacagggtgtatag

SEQ ID NO: 26 - DNA, 30 bp, Artificial Sequence
  rs298898-1st
acgttggatgatagtgtagtgagtgctatg

SEQ ID NO: 27 - DNA, 30 bp, Artificial Sequence
  rs2380657-2nd
acgttggatggctagggttgaaaaccaatg

SEQ ID NO: 28 - DNA, 30 bp, Artificial Sequence
  rs2380657-1st
acgttggatggaatatgagcacaacacacg

SEQ ID NO: 29 - DNA, 30 bp, Artificial Sequence
  rs2180770-2nd
acgttggatgcacttgtcacaaactctagg

SEQ ID NO: 30 - DNA, 30 bp, Artificial Sequence
  rs2180770-1st
acgttggatgaaccacagtgagcatggaag

SEQ ID NO: 31 - DNA, 30 bp, Artificial Sequence
  rs58616-2nd
acgttggatgtaggcagaaaagggctgaag

SEQ ID NO: 32 - DNA, 31 bp, Artificial Sequence
  rs58616-1st
acgttggatgcccttctgctttaacactatc

SEQ ID NO: 33 - DNA, 30 bp, Artificial Sequence
  rs265005-2nd
acgttggatgatcaggcacaatctctaccc

SEQ ID NO: 34 - DNA, 30 bp, Artificial Sequence
  rs265005-1st
acgttggatgacacaaagctaccactgcac

SEQ ID NO: 35 - DNA, 29 bp, Artificial Sequence
  rs1259859-2nd
acgttggatggccaattttatagaaactc

SEQ ID NO: 36 - DNA, 30 bp, Artificial Sequence
  rs1259859-1st
acgttggatgtagtatcaaggttttctggc

SEQ ID NO: 37 - DNA, 30 bp, Artificial Sequence
  rs1549944-2nd
acgttggatgtgtcacatatgctggccttg

SEQ ID NO: 38 - DNA, 30 bp, Artificial Sequence
  rs1549944-1st
acgttggatgctctcttgaagaaggtgcag

SEQ ID NO: 39 - DNA, 30 bp, Artificial Sequence
  rs1028330-2nd
acgttggatgttttcgggcagtgaagagac

SEQ ID NO: 40 - DNA, 30 bp, Artificial Sequence
  rs1028330-1st
acgttggatgctctacatctgtgggtctag

SEQ ID NO: 41 - DNA, 29 bp, Artificial Sequence
  rs1390272-2nd
acgttggatgcctttgatatttgttccac

SEQ ID NO: 42 - DNA, 30 bp, Artificial Sequence
  rs1390272-1st
acgttggatgcaggatagtctactatgtgc

SEQ ID NO: 43 - DNA, 30 bp, Artificial Sequence
  rs1434199-2nd
acgttggatgggcatagggagctgaatcaa

SEQ ID NO: 44 - DNA, 30 bp, Artificial Sequence
  rs1434199-1st
acgttggatgcacctctgccccctaatttc

SEQ ID NO: 45 - DNA, 30 bp, Artificial Sequence
  rs464221-2nd
acgttggatgtgaggacttgggattaggac

SEQ ID NO: 46 - DNA, 30 bp, Artificial Sequence
  rs464221-1st
acgttggatgaggcagcagcagaagtttag

SEQ ID NO: 47 - DNA, 30 bp, Artificial Sequence
  rs1522307-2nd
acgttggatgtagggtccagaaatgtgttg

SEQ ID NO: 48 - DNA, 30 bp, Artificial Sequence
  rs1522307-1st
acgttggatgggagaagcaagccatagatg

SEQ ID NO: 49 - DNA, 16 bp, Artificial Sequence
  rs248205-UEP
aaagctccaacacact

SEQ ID NO: 50 - DNA, 17 bp, Artificial Sequence
  rs248205-EXT1
aaagctccaacacactc

SEQ ID NO: 51 - DNA, 17 bp, Artificial Sequence
  rs248205-EXT2
aaagctccaacacactg

SEQ ID NO: 52 - DNA, 16 bp, Artificial Sequence
  rs2051068-UEP
gagcgcacaggtatag

SEQ ID NO: 53 - DNA, 17 bp, Artificial Sequence
  rs2051068-EXT1
gagcgcacaggtataga

SEQ ID NO: 54 - DNA, 17 bp, Artificial Sequence
  rs2051068-EXT2
gagcgcacaggtatagg

SEQ ID NO: 55 - DNA, 17 bp, Artificial Sequence
  rs1950501-UEP
gtgggtacaaaggtcaa

SEQ ID NO: 56 - DNA, 18 bp, Artificial Sequence
  rs1950501-EXT1
gtgggtacaaaggtcaac

SEQ ID NO: 57 - DNA, 18 bp, Artificial Sequence
  rs1950501-EXT2
gtgggtacaaaggtcaag

SEQ ID NO: 58 - DNA, 17 bp, Artificial Sequence
  rs1952966-UEP
cttggctgaagcaatac

SEQ ID NO: 59 - DNA, 18 bp, Artificial Sequence
  rs1952966-EXT1
cttggctgaagcaataca

SEQ ID NO: 60 - DNA, 18 bp, Artificial Sequence
  rs1952966-EXT2
cttggctgaagcaatacg

SEQ ID NO: 61 - DNA, 17 bp, Artificial Sequence
  AMG_mid100-UEP
tggaccacttgagaaac

SEQ ID NO: 62 - DNA, 18 bp, Artificial Sequence
  AMG_mid100-EXT1
tggaccacttgagaaacc

SEQ ID NO: 63 - DNA, 18 bp, Artificial Sequence
  AMG_mid100-EXT2
tggaccacttgagaaaca

SEQ ID NO: 64 - DNA, 18 bp, Artificial Sequence
  rs1385306-UEP
tttggctcatctgttctc

SEQ ID NO: 65 - DNA, 19 bp, Artificial Sequence
  rs1385306-EXT1
tttggctcatctgttctcc

SEQ ID NO: 66 - DNA, 19 bp, Artificial Sequence
  rs1385306-EXT2
tttggctcatctgttctcg

SEQ ID NO: 67 - DNA, 19 bp, Artificial Sequence
  rs1365740-UEP
cacctttttcctcttcatt

SEQ ID NO: 68 - DNA, 20 bp, Artificial Sequence
  rs1365740-EXT1
cacctttttcctcttcattg

SEQ ID NO: 69 - DNA, 20 bp, Artificial Sequence
  rs1365740-EXT2
cacctttttcctcttcattt

SEQ ID NO: 70 - DNA, 19 bp, Artificial Sequence
  rs2016207-UEP
agcacagaatcctttagaa

SEQ ID NO: 71 - DNA, 20 bp, Artificial Sequence
  rs2016207-EXT1
agcacagaatcctttagaac

SEQ ID NO: 72 - DNA, 20 bp, Artificial Sequence
  rs2016207-EXT2
agcacagaatcctttagaat

SEQ ID NO: 73 - DNA, 20 bp, Artificial Sequence
  rs1571256-UEP
tgcctctcagtactctagtc

SEQ ID NO: 74 - DNA, 21 bp, Artificial Sequence
  rs1571256-EXT1
tgcctctcagtactctagtca

SEQ ID NO: 75 - DNA, 21 bp, Artificial Sequence
  rs1571256-EXT2
tgcctctcagtactctagtcg

SEQ ID NO: 76 - DNA, 20 bp, Artificial Sequence
  rs1350836-UEP
ccacctcaaagggatattaa

SEQ ID NO: 77 - DNA, 21 bp, Artificial Sequence
  rs1350836-EXT1
ccacctcaaagggatattaac

SEQ ID NO: 78 - DNA, 21 bp, Artificial Sequence
  rs1350836-EXT2
ccacctcaaagggatattaat

SEQ ID NO: 79 - DNA, 20 bp, Artificial Sequence
  rs120434-UEP
gggttggcaacatggttaag

SEQ ID NO: 80 - DNA, 21 bp, Artificial Sequence
  rs120434-EXT1
gggttggcaacatggttaagc

SEQ ID NO: 81 - DNA, 21 bp, Artificial Sequence
  rs120434-EXT2
gggttggcaacatggttaagg

SEQ ID NO: 82 - DNA, 21 bp, Artificial Sequence
  rs2347790-UEP
ccccgatgtgcgtatgcctta

SEQ ID NO: 83 - DNA, 22 bp, Artificial Sequence
  rs2347790-EXT1
ccccgatgtgcgtatgccttaa

SEQ ID NO: 84 - DNA, 22 bp, Artificial Sequence
  rs2347790-EXT2
ccccgatgtgcgtatgccttag

SEQ ID NO: 85 - DNA, 21 bp, Artificial Sequence
  rs298898-UEP
gtgagtgctatgatcattatc

SEQ ID NO: 86 - DNA, 22 bp, Artificial Sequence
  rs298898-EXP1
gtgagtgctatgatcattatcc

SEQ ID NO: 87 - DNA, 22 bp, Artificial Sequence
  rs298898-EXP2
gtgagtgctatgatcattatct

SEQ ID NO: 88 - DNA, 22 bp, Artificial Sequence
  rs2380657-UEP
tggaacaacacacgtttttagt

SEQ ID NO: 89 - DNA, 23 bp, Artificial Sequence
  rs2380657-EXT1
tggaacaacacacgtttttagtc

SEQ ID NO: 90 - DNA, 23 bp, Artificial Sequence
  rs2380657-EXT2
tggaacaacacacgtttttagtt

SEQ ID NO: 91 - DNA, 23 bp, Artificial Sequence
  rs2180770-UEP
ccaaatataaccttgatcctctg

SEQ ID NO: 92 - DNA, 24 bp, Artificial Sequence
  rs2180770-EXT1
ccaaatataaccttgatcctctga

SEQ ID NO: 93 - DNA, 24 bp, Artificial Sequence
  rs2180770-EXT2
ccaaatataaccttgatcctctgg

SEQ ID NO: 94 - DNA, 23 bp, Artificial Sequence
  rs58616-UEP
tctgctttaacactatcagggta

SEQ ID NO: 95 - DNA, 24 bp, Artificial Sequence
  rs58616-EXT1
tctgctttaacactatcagggtac

SEQ ID NO: 96 - DNA, 24 bp, Artificial Sequence
  rs58616-EXT2
tctgctttaacactatcagggtat

SEQ ID NO: 97 - DNA, 23 bp, Artificial Sequence
  rs265005-UEP
tttatgctcaactggactataaa

SEQ ID NO: 98 - DNA, 24 bp, Artificial Sequence
  rs265005-EXT1
tttatgctcaactggactataaaa

SEQ ID NO: 99 - DNA, 24 bp, Artificial Sequence
  rs265005-EXT2
tttatgctcaactggactataaag

SEQ ID NO: 100 - DNA, 23 bp, Artificial Sequence
  rs1259859-UEP
gatgggaggtgatccttcttata

SEQ ID NO: 101 - DNA, 24 bp, Artificial Sequence
  rs1259859-EXT1
gatgggaggtgatccttcttatag

SEQ ID NO: 102 - DNA, 24 bp, Artificial Sequence
  rs1259859-EXT2
gatgggaggtgatccttcttatat

SEQ ID NO: 103 - DNA, 24 bp, Artificial Sequence
  rs1549944-UEP
ggggaggaaagaaacactgatcca

SEQ ID NO: 104 - DNA, 25 bp, Artificial Sequence
  rs1549944-EXT1
ggggaggaaagaaacactgatccaa

SEQ ID NO: 105 - DNA, 25 bp, Artificial Sequence
  rs1549944-EXT2
ggggaggaaagaaacactgatccag

SEQ ID NO: 106 - DNA, 25 bp, Artificial Sequence
  rs1028330-UEP
ccactgacatgtatccaccattatg

SEQ ID NO: 107 - DNA, 26 bp, Artificial Sequence
  rs1028330-EXT1
ccactgacatgtatccaccattatga

SEQ ID NO: 108 - DNA, 26 bp, Artificial Sequence
  rs1028330-EXT2
ccactgacatgtatccaccattatgg

SEQ ID NO: 109 - DNA, 25 bp, Artificial Sequence
  rs1390272-UEP
gcttggtttttcttaacaagttcac

SEQ ID NO: 110 - DNA, 26 bp, Artificial Sequence
  rs1390272-EXT1
gcttggtttttcttaacaagttcaca

SEQ ID NO: 111 - DNA, 26 bp, Artificial Sequence
  rs1390272-EXT2
gcttggtttttcttaacaagttcacg

SEQ ID NO: 112 - DNA, 25 bp, Artificial Sequence
  rs1434199-UEP
gatttgaaggtctagaactttcatt

SEQ ID NO: 113 - DNA, 26 bp, Artificial Sequence
  rs1434199-EXT1
gatttgaaggtctagaactttcattc

SEQ ID NO: 114 - DNA, 26 bp, Artificial Sequence
  rs1434199-EXT2
gatttgaaggtctagaactttcattg

SEQ ID NO: 115 - DNA, 26 bp, Artificial Sequence
  rs464221-UEP
gtcagcagcagaagtttagacaatta

SEQ ID NO: 116 - DNA, 27 bp, Artificial Sequence
  rs464221-EXT1
gtcagcagcagaagtttagacaattac

SEQ ID NO: 117 - DNA, 27 bp, Artificial Sequence
  rs464221-EXT2
gtcagcagcagaagtttagacaattat

SEQ ID NO: 118 - DNA, 26 bp, Artificial Sequence
  rs1522307-UEP
tagaaagccatagatgaaaatacgga

SEQ ID NO: 119 - DNA, 27 bp, Artificial Sequence
  rs1522307-EXT1
tagaaagccatagatgaaaatacggac

SEQ ID NO: 120 - DNA, 27 bp, Artificial Sequence
  rs1522307-EXT2
tagaaagccatagatgaaaatacggat